European Patent Application EP 4 438 735 A1, published October 2, 2024. Title: Biocatalytic preparation of chemicals using cofactor depending enzymes. Applicant: CASCAT GmbH. The sequence listing filed with the application follows.

SEQUENCE LISTING (40 sequences)

SEQ ID NO: 1 - protein, 263 aa, Herbaspirillum seropedicae DSM 6445
MTAATTPAFEHALYRSLAGKRVVITGGGSGIGAALVEAFVGQGAQVCFLDIAAEPSQALVASLKDAPIAPRFFPCNLMNLEALRATFTEIETVMGGVDILINNAANDDRHKTADVTPAYWDERLAVNLRHQFFCAQAVLPGMRERKQGVILNFGSISWHLGLPYLTLYMTAKAGIEGMTHGMARDFGRDGVRVNAIIPGAIRTPRQTLLWHTPEEEAKILAAQCLPTRVDPHDVAALALFLSSDSGAKCTGREYYVDAGWLGA

SEQ ID NO: 2 - DNA, 792 bp, Herbaspirillum seropedicae DSM 6445
  source 1..792: mol_type = genomic DNA
atgaccgcagccaccacccccgcattcgaacacgccctctatcgcagcctcgccggcaagcgggtcgtcatcaccggcggcggcagcggcatcggcgcggccctggtggaagccttcgtcggacaaggcgcacaggtgtgcttcctggatatcgccgccgagccctcgcaggcgctggtggcgtcgctcaaggatgcgccgatcgcgccgcgcttcttcccctgcaacctgatgaacctggaagccttgcgcgccaccttcaccgagatcgaaacggtgatgggcggggtggacatcctcatcaacaacgccgccaatgatgaccgtcacaagaccgccgacgtcacgcccgcctattgggacgaacgcctggcggtcaacctgcgccaccagttcttctgcgcccaggccgtgctgccgggcatgcgcgagcgcaagcagggcgtgatcctcaatttcggctccatctcctggcatctcggcttgccttacctgaccctgtacatgaccgccaaggccggcatcgaaggcatgacccacggcatggcgcgcgactttggccgcgatggcgtgcgggtcaacgccatcattcccggcgccatccgtaccccgcgccagaccctgctctggcacacccccgaagaagaggcgaaaatcctggctgcgcaatgcctgcctacccgtgtcgatccgcatgatgtcgctgccctggcgctgttcctgtcctccgacagcggcgccaagtgcaccggccgcgagtactacgtcgatgccggctggctgggcgcgtaa

SEQ ID NO: 3 - protein, 261 aa, Herbaspirillum seropedicae DSM 6445
MSNTPQNVQLASFPSLKGKRVFITGGGTGIGAAIVEAFAQQGAHVAFVDIATEASEALCNEVAAAGHPKPLFRHCDLRDIPAFQATIAELQAQLGDFDVLVNNAANDQRHKLEEVTLEYWNDRIAINQRPSFFAVQSVVEGMKRRGGGSIINFSSISWHQSGGGFPVYTTAKASTLGLTRGLARDLGPHKIRVNTVTPGWVMTERQIKLWLDEEGKKAIARNQCLQGDLLPWHLARMVLFLAADDSAMCTAQEFIVDAGWV

SEQ ID NO: 4 - DNA, 786 bp, Herbaspirillum seropedicae DSM 6445
  source 1..786: mol_type = genomic DNA
atgagcaacactccccagaacgtgcaactggcgagcttccccagcttgaagggcaagcgcgtcttcatcaccggtggcggcaccggcattggcgcggccatcgtcgaagcgtttgcgcaacaaggtgcgcatgtggctttcgtcgatatcgccaccgaagccagcgaagcgctgtgcaacgaggtggccgcggccggtcaccccaagccgctgttccgccattgcgacctgcgcgacatcccggctttccaggccaccatcgccgaactgcaagcccagctgggcgatttcgacgtgctggtcaacaacgccgccaacgaccagcgccacaagctggaagaagtgacgctggaatactggaacgaccgcatcgccatcaatcagcgcccgtccttcttcgccgtgcagtcggtggtggaggggatgaagcgccgcggcggcggctccatcatcaacttcagttcgatcagctggcaccagtccggcggcggcttcccggtctataccacggccaaggcctcgaccctgggcttgacccgtggcctggcgcgcgacctcggtccgcacaagatccgcgtcaataccgtcacgccaggctgggtcatgaccgagcgccagatcaagttgtggctggacgaagagggcaagaaggccatcgcccgcaaccagtgcctgcagggcgacctgttgccgtggcacctggcgcgcatggtgctgttcctggctgctgacgatagcgccatgtgcaccgcgcaggaattcatcgtcgatgccggttgggtctaa

SEQ ID NO: 5 - protein, 295 aa, Noviherbaspirillum massiliense JC206 DSM25712
MKTPECVWDTHAQLGEGPLWSSKAQALYWVDILGRRLHRYSPWEGQRSWAFEEEISAVAERAGGNGLIVTLRRGFAFFDPASGQLEHLIQPETDLPNNRFNDGKCDARGRFWAGSMDFEGRQTSGSLYRLSADLACVRMDGGYAVTNGPAWSADNRTMYFNDSANGRVYAFDFDLDAGGLSNKRLFLQFPAEEGVPDGMTTDAEGGLWIAHWGAGKLTRHDAAGKVLHAIDLPCSQVSSCAFGGPDMKTLFITTALTGLSNEQLAREPLAGGLFAVDLDIAGVPANTFRSELTSA

SEQ ID NO: 6 - DNA, 888 bp, Noviherbaspirillum massiliense JC206 DSM25712
  source 1..888: mol_type = genomic DNA
atgaagactccggagtgtgtctgggacactcatgcccaactaggcgaaggcccgctctggtcatccaaggcgcaagccttgtactgggtcgacatcctcgggcgacgcctgcatcgctattcgccatgggaggggcagcgcagctgggccttcgaggaagaaatttcagcagtagcggaacgcgcaggggggaatgggttgatcgttaccctgcgccgcggcttcgccttcttcgaccccgctagcgggcaactggagcatctgatccagccggagacggacctgccgaacaatcgtttcaatgacggcaaatgcgatgcgcgcggccggttctgggccggcagcatggatttcgagggcaggcaaacaagtggctccctgtaccgtctttcggccgacctcgcctgtgtgcgcatggatggcggctatgcggtgaccaacggccccgcatggtctgccgacaatcggacgatgtatttcaacgacagtgcgaacggccgtgtctatgccttcgacttcgaccttgatgccggcggcttgtccaacaagcgcctgttcctgcaattcccggcggaggaaggcgtcccggacggcatgaccaccgatgcggaaggcgggctctggatcgcgcactggggcgcgggaaagctgactcggcatgatgcggctggcaaggtgctgcatgcgatcgaccttccctgcagccaggtatcgagctgcgccttcggcggaccggacatgaaaaccctgttcatcaccactgcactcaccggactgtcgaacgaacaactggcgcgcgagccgctggctggcggattgttcgccgtcgatctcgatattgccggcgtacccgccaatactttccgaagcgagctgacatccgcatga

SEQ ID NO: 7 - protein, 575 aa, Paralcaligenes ureilyticus DSM 24591
MSDKEKPVRRSQAWFGRLDRDGFIYRSWMKNRGIPHDQFDGRPVIGICNTFSELTPCNSHFRTLAEQVKIGVWESGGFPLEFPVMSLGETMLRPTAMLFRNLASMDVEESIRGNPLDGVVLLMGCDKTTPSLMMGAASCDLPTIGVSGGPMLSGKFRGRELGSGTDVWKMSEEVRAGQMSQEEFFEAESCMHRSHGHCMTMGTASTMASMVEALGMSLPGNAAIPAVDARRNLLARASGRRIVQMVKDDLVMSKILTRQAFENAIRVNAAIGGSTNAVIHLLAIAGRIGVDLTLADWDALGHKLPCLVDLQPSGTHLMEDFYYAGGVPAVIRELGDVIARDALTVNGQTLWDNCKDAPNWNREVIHAFNEPFKTEAGIAVLRGNLCPDGAVIKPSAATPALLKHKGRAVVFENSEHMHERMDDENLDVDENCVLVLKNCGPRGYPGMAEAGNMPLPPKILRKGITDMVRVSDARMSGTAYGTVVLHVAPEAAAGGPLALVQDGDIIELDVAARKLHLHVSDEELARRREAWQAPPAPMARGWVKLYVEHVQQANLGADLDFLRGKSGAGIPKDNH

SEQ ID NO: 8 - DNA, 1728 bp, Paralcaligenes ureilyticus DSM 24591
  source 1..1728: mol_type = genomic DNA
atgagtgacaaagaaaagcctgtgcgtcgcagccaggcctggttcggacggcttgaccgcgacggtttcatctaccgttcgtggatgaagaatcgaggcatcccgcacgatcagttcgacggtcgcccggtgattggcatttgcaatactttctctgaactgacgccgtgcaattcgcatttccgcaccttggccgagcaggtcaagatcggggtttgggagtcgggcggcttccctctcgagtttccggtcatgtcgctgggcgagacgatgttgcggcctacggccatgctgtttcgcaacctggccagcatggacgtcgaggaatcgatacgcggcaatccgttggatggcgtcgtattgctgatgggctgcgacaaaacgacgccttcgctcatgatgggggcggcgtcctgcgacctgcccactatcggtgtgtcgggcggtcccatgcttagcggcaagtttcgaggccgcgaactgggttcaggcaccgacgtctggaagatgtctgaagaagttcgcgccgggcaaatgtcgcaggaagaatttttcgaagcggaaagctgcatgcatcgctcgcatgggcattgcatgacgatgggtacggcatccacgatggccagcatggtggaagcgctgggcatgagcctgcctggcaacgcggcgattcccgccgtggatgcgcgccgcaatctgctcgcgcgcgcttcgggccggcgcattgtgcagatggtcaaagatgatctggtcatgtcgaaaatcctgacgcgccaggcctttgaaaacgccatccgcgtgaacgccgctatcggtggctcgaccaacgcggtgattcatctgttggcgattgcggggcgtatcggggttgacctgacgcttgccgactgggatgcgctcggccacaaattgccgtgcctggttgatctgcagccttcgggcactcatctgatggaagacttttattatgcgggcggcgtgcccgccgtgatccgcgagctgggcgatgtcattgcccgcgatgccctgacggtgaatggccagaccctgtgggataactgcaaggatgcgccaaactggaatcgcgaggtcatccatgcctttaacgagcctttcaagaccgaggcggggatagccgtactgcgtggcaacctatgccccgatggggccgtcatcaaaccttcggccgccacgccggccctgctcaagcacaagggccgcgcggtcgtgttcgaaaacagcgaacatatgcacgagcgcatggacgatgaaaacctggacgtcgacgagaattgcgtgctggttttgaagaattgcgggccccgcggctatccgggtatggccgaagccggcaatatgccgctgccgccgaaaatcctgcgcaaaggcatcaccgatatggtccgggtgtccgacgcccgcatgagcggcaccgcgtatggcacggtggttctgcatgtggcccccgaggccgccgcgggcggccctttggcgctggtgcaggacggcgacatcatcgaactggatgtggccgcgcgcaagctgcatttgcatgtgtccgatgaagagctcgcacgccgccgcgaggcatggcaagcgccgccggcgcccatggcgcgcggctgggtcaagctttatgtcgagcatgtgcagcaagccaatctgggcgccgaccttgattttctgcgaggtaaaagcggcgcgggcatacccaaagacaatcactga

SEQ ID NO: 9 - protein, 550 aa, Lactococcus lactis
MASMYTVGDYLLDRLHELGIEEIFGVPGDYNLQFLDQIISREDMKWIGNANELNASYMADGYARTKKAAAFLTTFGVGELSAINGLAGSYAENLPVVEIVGSPTSKVQNDGKFVHHTLADGDFKHFMKMHEPVTAARTLLTAENATYEIDRVLSQLLKERKPVYINLPVDVAAAKAEKPALSLEKESSTTNTTEQVILSKIEESLKNAQKPVVIAGHEVISFGLEKTVTQFVSETKLPITTLNFGKSAVDESLPSFLGIYNGKLSEISLKNFVESADFILMLGVKLTDSSTGAFTHHLDENKMISLNIDEGIIFNKVVEDFDFRAVVSSLSELKGIEYEGQYIDKQYEEFIPSSAPLSQDRLWQAVESLTQSNETIVAEQGTSFFGASTIFLKSNSRFIGQPLWGSIGYTFPAALGSQIADKESRHLLFIGDGSLQLTVQELGLSIREKLNPICFIINNDGYTVEREIHGPTQSYNDIPMWNYSKLPETFGATEDRVVSKIVRTENEFVSVMKEAQADVNRMYWIELVLEKEDAPKLLKKMGKLFAEQNK

SEQ ID NO: 10 - DNA, 1644 bp, Lactococcus lactis
  source 1..1644: mol_type = genomic DNA
atgtatacagtaggagattacctgttagaccgattacacgagttgggaattgaagaaatttttggagttcctggtgactataacttacaatttttagatcaaattatttcacgcgaagatatgaaatggattggaaatgctaatgaattaaatgcttcttatatggctgatggttatgctcgtactaaaaaagctgccgcatttctcaccacatttggagtcggcgaattgagtgcgatcaatggactggcaggaagttatgccgaaaatttaccagtagtagaaattgttggttcaccaacttcaaaagtacaaaatgacggaaaatttgtccatcatacactagcagatggtgattttaaacactttatgaagatgcatgaacctgttacagcagcgcggactttactgacagcagaaaatgccacatatgaaattgaccgagtactttctcaattactaaaagaaagaaaaccagtctatattaacttaccagtcgatgttgctgcagcaaaagcagagaagcctgcattatctttagaaaaagaaagctctacaacaaatacaactgaacaagtgattttgagtaagattgaagaaagtttgaaaaatgcccaaaaaccagtagtgattgcaggacacgaagtaattagttttggtttagaaaaaacggtaactcagtttgtttcagaaacaaaactaccgattacgacactaaattttggtaaaagtgctgttgatgaatctttgccctcatttttaggaatatataacgggaaactttcagaaatcagtcttaaaaattttgtggagtccgcagactttatcctaatgcttggagtgaagcttacggactcctcaacaggtgcattcacacatcatttagatgaaaataaaatgatttcactaaacatagatgaaggaataattttcaataaagtggtagaagattttgattttagagcagtggtttcttctttatcagaattaaaaggaatagaatatgaaggacaatatattgataagcaatatgaagaatttattccatcaagtgctcccttatcacaagaccgtctatggcaggcagttgaaagtttgactcaaagcaatgaaacaatcgttgctgaacaaggaacctcattttttggagcttcaacaattttcttaaaatcaaatagtcgttttattggacaacctttatggggttctattggatatacttttccagcggctttaggaagccaaattgcggataaagagagcagacaccttttatttattggtgatggttcacttcaacttaccgtacaagaattaggactatcaatcagagaaaaactcaatccaatttgttttatcataaataatgatggttatacagttgaaagagaaatccacggacctactcaaagttataacgacattccaatgtggaattactcgaaattaccagaaacatttggagcaacagaagatcgtgtagtatcaaaaattgttagaacagagaatgaatttgtgtctgtcatgaaagaagcccaagcagatgtcaatagaatgtattggatagaactagttttggaaaaagaagatgcgccaaaattactgaaaaaaatgggtaaattatttgctgagcaaaataaatag

SEQ ID NO: 11 - protein, 339 aa, Escherichia coli
MSMIKSYAAKEAGGELEVYEYDPGELRPQDVEVQVDYCGICHSDLSMIDNEWGFSQYPLVAGHEVIGRVVALGSAAQDKGLQVGQRVGIGWTARSCGHCDACISGNQINCEQGAVPTIMNRGGFAEKLRADWQWVIPLPENIDIESAGPLLCGGITVFKPLLMHHITATSRVGVIGIGGLGHIAIKLLHAMGCEVTAFLNDPAKEQEVLAMGADKVVNSRDPQALKALAGQFDLIINTVNVSLDWQPYFEALTYGGNFHTVGAVLTPLSVPAFTLIAGDRSVSGSATGTPYELRKLMRFAARSKVAPTTELFPMSKINDAIQHVRDGKARYRVVLKADF

SEQ ID NO: 12 - DNA, 1020 bp, Escherichia coli
  source 1..1020: mol_type = other DNA
atgtcgatgataaaaagctatgccgcaaaagaagcgggcggcgaactggaagtttatgagtacgatcccggtgagctgaggccacaagatgttgaagtgcaggtggattactgcgggatctgccattccgatctgtcgatgatcgataacgaatggggattttcacaatatccgctggttgccgggcatgaggtgattgggcgcgtggtggcactcgggagcgccgcgcaggataaaggtttgcaggtcggtcagcgtgtcgggattggctggacggcgcgtagctgtggtcactgcgacgcctgtattagcggtaatcagatcaactgcgagcaaggtgcggtgccgacgattatgaatcgcggtggctttgccgagaagttgcgtgcggactggcaatgggtgattccactgccagaaaatattgatatcgagtccgccgggccgctgttgtgcggcggtatcacggtctttaaaccactgttgatgcaccatatcactgctaccagccgcgttggggtaattggtattggcgggctggggcatatcgctataaaacttctgcacgcaatgggatgcgaggtgacagcctttcttaatgatccggcgaaagagcaggaagtgctggcgatgggtgccgataaagtggtgaatagccgcgatccgcaggcactgaaagcactggcggggcagtttgatctcattatcaacaccgtcaacgtcagcctcgactggcagccctattttgaggcgctgacctatggcggtaatttccatacggtcggtgcggttctcacgccgctgtctgttccggcctttacgttaattgcgggcgatcgcagcgtctctggttctgctaccggcacgccttatgagctgcgtaagctgatgcgttttgccgcccgcagcaaggttgcgccgaccaccgaactgttcccgatgtcgaaaattaacgacgccatccagcatgtgcgcgacggtaaggcgcgttaccgcgtggtgttgaaagccgatttttga

SEQ ID NO: 13 - protein, 260 aa, Bacillus subtilis
MYPDLKGKVVAITGAASGLGKAMAIRFGKEQAKVVINYYSNKQDPNEVKEEVIKAGGEAVVVQGDVTKEEDVKNIVQTAIKEFGTLDIMINNAGLENPVPSHEMPLKDWDKVIGTNLTGAFLGSREAIKYFVENDIKGNVINMSSVHEVIPWPLFVHYAASKGGIKLMTKTLALEYAPKGIRVNNIGPGAINTPINAEKFADPKQKADVESMIPMGYIGEPEEIAAVAAWLASKEASYVTGITLFADGGMTLYPSFQAGR

SEQ ID NO: 14 - DNA, 786 bp, Bacillus subtilis
  source 1..786: mol_type = other DNA
atgtatccggatttaaaaggaaaagtcgtcgctattacaggagctgcttcagggctcggaaaggcgatggccattcgcttcggcaaggagcaggcaaaagtggttatcaactattatagtaataaacaagatccgaacgaggtaaaagaagaggtcatcaaggcgggcggtgaagctgttgtcgtccaaggagatgtcacgaaagaggaagatgtaaaaaatatcgtgcaaacggcaattaaggagttcggcacactcgatattatgattaataatgccggtcttgaaaatcctgtgccatctcacgaaatgccgctcaaggattgggataaagtcatcggcacgaacttaacgggtgcctttttaggaagccgtgaagcgattaaatatttcgtagaaaacgatatcaagggaaatgtcattaacatgtccagtgtgcacgaagtgattccttggccgttatttgtccactatgcggcaagtaaaggcgggataaagctgatgacaaagacattagcgttggaatacgcgccgaagggcattcgcgtcaataatattgggccaggtgcgatcaacacgccaatcaatgctgaaaaattcgctgaccctaaacagaaagctgatgtagaaagcatgattccaatgggatatatcggcgaaccggaggagatcgccgcagtagcagcctggcttgcttcgaaggaagccagctacgtcacaggcatcacgttattcgcggacggcggtatgacactctatccttcattccaggcaggccgcggttaa

SEQ ID NO: 15 - protein, 261 aa, Bacillus subtilis
MYPDLKGKVVAITGAASGLGKAMAIRFGKEQAKVVINYYSNKQDAEEVKEEVIKAGGEAVVVQGDVTKEEDVKNIVQTAIKEFGTLDIMINNAGLENPVPSHEMPLKDWDKVIGTNLTGAFLGSREAIKYFVENDIKGNVINMSSVHEVIPWPLYVHYAASKGGIKLMTKTLALEYAPKGIRVNNIGPGAINTPINAEKFADPKQKADVESMIPMGYIGEPEEIAAAAAFLASKEASYVTGITLFADGGMTLYPSFQAGRG

SEQ ID NO: 16 - DNA, 786 bp, Bacillus subtilis
  source 1..786: mol_type = other DNA
atgtatccggatttaaaaggaaaagtcgtcgctattacaggagctgcttcagggctcggaaaggcgatggccattcgcttcggcaaggagcaggcaaaagtggttatcaactattatagtaataaacaagatgcggaagaggtaaaagaagaggtcatcaaggcgggcggtgaagctgttgtcgtccaaggagatgtcacgaaagaggaagatgtaaaaaatatcgtgcaaacggcaattaaggagttcggcacactcgatattatgattaataatgccggtcttgaaaatcctgtgccatctcacgaaatgccgctcaaggattgggataaagtcatcggcacgaacttaacgggtgcctttttaggaagccgtgaagcgattaaatatttcgtagaaaacgatatcaagggaaatgtcattaacatgtccagtgtgcacgaagtgattccttggccgttatatgtccactatgcggcaagtaaaggcgggataaagctgatgacaaagacattagcgttggaatacgcgccgaagggcattcgcgtcaataatattgggccaggtgcgatcaacacgccaatcaatgctgaaaaattcgctgaccctaaacagaaagctgatgtagaaagcatgattccaatgggatatatcggcgaaccggaggagatcgccgcagcggcagcctttcttgcttcgaaggaagccagctacgtcacaggcatcacgttattcgcggacggcggtatgacactctatccttcattccaggcaggccgcggttaa

SEQ ID NO: 17 - protein, 265 aa, Agrobacterium tumefaciens C58
MKRLLVTGAAGQLGRVMRERLAPMAEILRLADLSPLDPAGPNEECVQCDLADANAVNAMVAGCDGIVHLGGISVEKPFEQILQGNIIGLYNLYEAARAHGQPRIVFASSNHTIGYYPQTERLGPDVPARPDGLYGVSKCFGENLARMYFDKFGQETALVRIGSCTPEPNNYRMLSTWFSHDDFVSLIEAVFRAPVLGCPVVWGASANDAGWWDNSHLGFLGWKPKDNAEAFRRHITETTPPPDPNDALVRFQGGTFVDNPIFKQS

SEQ ID NO: 18 - DNA, 798 bp, Agrobacterium tumefaciens C58
  source 1..798: mol_type = other DNA
atgaaacgtctgctggttaccggtgcagccggtcagctgggtcgtgttatgcgtgaacgtctggcaccgatggcagaaattctgcgtctggcagatctgtctccgctggatccggctggtccgaatgaagaatgtgttcagtgtgatctggcagatgcaaatgcagttaatgcaatggttgccggttgtgatggtattgttcatctgggtggcattagcgttgaaaaaccgtttgagcagattctgcagggtaacattattggcctgtataatctgtatgaagcagcacgtgcacatggtcagcctcgtattgtttttgcaagcagcaaccataccattggttattatccgcagaccgaacgtctgggtccggatgttccagcacgtcctgatggtctgtatggtgttagcaaatgctttggtgaaaatctggcacgcatgtattttgataaatttggccaggaaaccgcactggttcgtattggtagctgtacaccggaaccgaataattatcgtatgctgagcacctggtttagccatgatgattttgttagcctgattgaagcagtttttcgtgcaccggttctgggttgtccggttgtttggggtgcaagcgcaaatgatgccggttggtgggataatagccatctgggttttctgggttggaaaccgaaagataatgcagaagcctttcgtcgtcatattaccgaaaccacaccgcctccggatccgaatgatgccctggttcgttttcagggtggcacctttgttgataacccgatctttaaacagagctaa

SEQ ID NO: 19 - protein, 442 aa, Actinobacillus succinogenes 130Z
MSTPIITEMQVIPVAGHDSMLLNLSGAHSPYFTRNIVILKDNSGNTGVGEVPGGEKIRQTLEDAKPLVIGKTLGEYKNVMNTVRQTFNDHDAGGRGLQTFDLRTTIHVVTAIEAAMLDLLGQFLGVTVASLLGDGQQRDAVEMLGYLFFIGDRKKTTLAYQNQENDPCDWYRVRHEEAMTPESVVRLAEAAYEKYGFNDFKLKGGVLDGFEEAEAVTALAKRFPDARITLDPNGAWSLDEAVKIGKQLKGVLAYAEDPCGAEQGYSGREIMAEFRRATGLPTATNMIATDWRQMGHTISLQSVDIPLADPHFWTMQGSIRVAQMCHEWGLTWGSHSNNHFDISLAMFTHVAAAAPGDITAIDTHWIWQEGNQRLTKEPFQIKGGLVEVPKKPGLGVELDMDQVMKANELYKSMGLGARDDAMAMQFLIPGWKFDNKKPCLVR

SEQ ID NO: 20 - DNA, 1329 bp, Actinobacillus succinogenes 130Z
  source 1..1329: mol_type = other DNA
atgagcaccccgattattaccgaaatgcaagttattccggttgccggtcatgatagcatgctgctgaatctgagcggtgcacatagcccgtattttacccgcaacatcgtgattctgaaagataacagcggtaataccggtgttggtgaagttccgggtggtgaaaaaattcgtcagaccctggaagatgcaaaaccgctggttattggtaaaaccctgggcgaatataaaaatgtgatgaataccgtgcgtcagacctttaatgatcatgatgccggtggtcgtggcctgcagacatttgatctgcgtaccaccattcatgttgttaccgcaattgaagcagcaatgctggatctgctgggtcagtttctgggtgttaccgttgcaagcctgctgggtgatggtcagcagcgtgatgcagttgaaatgctgggctacctgttttttatcggcgatcgtaaaaaaaccaccctggcctatcagaatcaggaaaatgatccttgcgattggtatcgtgttcgtcatgaagaagcaatgacaccggaaagcgttgttcgtctggccgaagcagcctatgaaaaatatggctttaatgattttaaactgaaaggtggtgtgctggatggttttgaagaagcagaagcagttaccgcactggcaaaacgttttccggatgcacgtattaccctggatccgaatggtgcgtggagcctggatgaagcagttaaaatcggtaaacagctgaaaggtgttctggcctatgccgaagatccgtgtggtgcagaacagggttatagcggtcgtgaaattatggcagaatttcgtcgtgcaaccggtctgccgaccgcaaccaatatgattgcaaccgattggcgtcagatgggtcataccattagcctgcagagcgttgatattccgctggcagatccgcatttttggaccatgcagggtagcattcgtgttgcacagatgtgtcatgaatggggtctgacctggggtagccatagcaacaaccattttgatatcagcctggccatgtttacccatgttgcagcagcagcaccgggtgatattaccgccattgatacccattggatttggcaggaaggtaatcagcgtctgaccaaagaaccgtttcagattaaaggtggtctggttgaagttccgaaaaaaccgggtctgggtgttgaactggatatggatcaggtgatgaaagccaacgaactgtataaaagcatgggtctgggtgcacgtgatgatgcaatggcaatgcagtttctgattccgggttggaaatttgataacaaaaaaccgtgcctggtgcgttaa

SEQ ID NO: 21 - protein, 303 aa, Acinetobacter baylyi ADP1
MDALELKNIVSDGLLSFPVTDFDQNGDFNAASYAKRLEWLAPYGASALFAAGGTGEFFSLTGDEYSDVIKTAVDACKGSVPIIAGAGGPTRQAILQAQEAERLGAHGILLMPHYLTEASQEGLVEHVKQVCNAVNFGVIFYNRSVSKLNVDSLQQLVESCPNLIGFKDSSGQIDMMTEVVQTLGDRLSYLGGLPTAEIFAAPYKALGSPVYSSAVFNFIPKTAMEFYNALRNDDFATTQRLIRDFFLPLIKIRNRKSGYAVSMVKAGAKIVGHDAGPVRPPLSDLTPQDYEDLAALIATLGPQ

SEQ ID NO: 22 - DNA, 912 bp, Acinetobacter baylyi ADP1
  source 1..912: mol_type = other DNA
atggatgccctggaactgaaaaatattgtgtctgatggtctgctgagctttccggttaccgattttgatcagaatggcgattttaatgcagcaagctatgcaaaacgtctggaatggctggcaccgtatggtgcaagcgcactgtttgcagccggtggcacaggtgaattttttagcctgaccggtgatgaatattccgatgtgatcaaaaccgcagttgatgcatgtaaaggtagcgttccgattattgccggtgccggtggtccgacccgtcaggcaattctgcaggcacaggaagcagaacgtctgggagcacatggtattctgctgatgccgcattatctgaccgaagcaagccaggaaggtctggttgaacacgttaaacaggtgtgcaatgccgttaattttggcgtgatcttttataatcgtagcgtgagcaaactgaatgttgatagcctgcagcagctggttgaaagctgtccgaatctgattggttttaaagatagcagcggtcagattgatatgatgaccgaagttgttcagaccctgggtgatcgtctgagctatctgggtggtctgccgaccgcagaaatttttgcagcaccgtataaagcactgggttctccggtttatagcagcgcagtgtttaactttattccgaaaaccgccatggaattttataatgccctgcgcaatgatgattttgcaaccacccagcgtctgattcgtgatttttttctgccgctgattaaaattcgtaaccgtaaaagcggttatgcagttagcatggttaaagccggtgcaaaaattgttggtcatgatgccggtccggttcgtccgcctctgagcgatctgacaccgcaggattatgaagatctggcagcactgattgcaaccctgggtccgcagtaa

SEQ ID NO: 23 - protein, 480 aa, Variovorax paradoxus B4
MTATYTDTRLLIDNEWVDATGGKTLDVVNPATGKVIGKVAHASIADLDRALAAAQRGFDKWRNTPANERAAVMRRAAGLIRERAGDIAKLLTQEQGKPLAEAKGETLAAADIIEWFADEGRRVYGRIVPSRNLAAQQLVLKEPLGPVAAFTPWNFPINQIVRKLGAALATGCSFLVKAPEETPASPAALLQAFVDAGIPPGTVGLVFGNPAEISNYLIAHPIIRKVTFTGSTPVGKQLAALAGSHMKRVTMELGGHAPVIVAEDADVALAVKAAGAAKFRNAGQVCISPTRFLVHNSLREEFARTLVKYTEGLKLGDGLAEGTTIGPLANARRLTAMAYVLEDARKKGATVAAGGERVGDSGNFFAPTVLTDVPLDADVFNNEPFGPIAAIRGFDTLEEAIAEANRLPFGLAGYAFTKSIKSAHLLSQKLELGMLWINQPATPSPEMPFGGVKDSGYGSEGGPEALEAYLNTKAVSILGV

SEQ ID NO: 24 - DNA, 1444 bp, Variovorax paradoxus B4
  source 1..1444: mol_type = genomic DNA
atgaccgccacctacaccgacacccgcctgctgatcgacaacgaatgggtcgacgccaccggcggcaagacgctggacgtcgtgaaccccgccaccggcaaagtcatcggcaaggtggcgcatgccagcatcgccgacctggaccgcgccctggccgccgcccagcgcggcttcgacaaatggcgcaacacccccgccaacgagcgcgccgccgtcatgcgccgcgcagccggcctcatccgcgaacgcgccggcgacatcgccaagctgctgacgcaagagcagggcaagccgctcgccgaagccaagggcgagaccctggccgccgccgacatcatcgaatggttcgccgacgaaggccgccgcgtctacggccgcatcgtgccctcgcggaacctggccgcgcagcagctcgtgctcaaggagccgctcggccccgtcgcagcgttcacgccgtggaacttcccgatcaaccagatcgtgcgcaagctcggcgcagcgctggccaccggctgctcgttcctggtgaaggcgcccgaagaaaccccggcgtcccccgccgcgctgctgcaggctttcgtcgacgcaggcattccgcccggcaccgtcggcctcgtgttcggcaaccccgctgaaatctcgaactacctcattgcccacccgatcatccgcaaggtcaccttcaccggctcgaccccggtcggcaagcagctggccgcgctggccggctcgcacatgaagcgcgtcacgatggagctgggcggccacgccccggtgatcgtggccgaagacgccgacgttgccctggccgtcaaggccgccggcgccgccaagttccgcaatgccggccaggtctgcatttcgccgacccgcttcctggtgcacaacagcctgcgcgaagagttcgcccgcacgctggtcaagtacaccgaaggcctgaagctcggcgacggcctcgccgaaggcaccaccatcggcccgctggccaacgcacgccgcctcaccgcgatggcctacgtgctggaagacgcgcgcaagaagggcgccacagtggcggccggcggcgaacgcgtcggcgactcgggcaactttttcgcgcccaccgtgctgaccgacgtgccgctggacgccgacgtgttcaacaacgagcccttcggccccatcgccgcgatccgtggcttcgacacgctcgaagaagcgatcgccgaagccaaccgcctgccattcggcctggccggctacgccttcaccaagtcgatcaagagcgcccacctgctgagccagaagctcgaactcggcatgctgtggatcaaccagcccgccaccccgtcgccggaaatgccgttcggcggcgtgaaggattcgggctacggttcggaaggcggccccgaggcgctcgaggcttacctgaacaccaaggccgtgtcgatcctcggcgtttaaa

SEQ ID NO: 25 - protein, 405 aa, Pseudomonas putida DSM 6125
MTDRTNANQPLPLSHDASVFDRGSWVGRVWLPEQGPAVVLVKAGAVYDISTHVATVSALLEVDDPVAYLRALPLAEPLIALPALLGNSDPTRRTPHQPWLLAPIDLQAVKAAGVTFATSLLERVVEEQAKGDPAKADAIRDTLASRIGADLSQIVPGSAQAEALRKVLVEQGLWSQYLEVGIGPDAEVFTKAQPLSAVGHGADIGIHPKSSWNNPEPEVVLAVSSNGSIKGAMLGNDVNLRDFEGRSALLLSKAKDNNASTALGPLLRLFDESFGLDDVRAAEVDLRVEGEDGFILSGRSSMRQISRDPQDLVQQTLNENHQYPDGLVLFLGTLFAPKQDRDQPGNGFTHKPGDVVSISNPQLGTLCNRVTTSDLAPQWDFGLRALIDNLGRRGLLEVAATARPL

SEQ ID NO: 26 - DNA, 1218 bp, Pseudomonas putida DSM 6125
  source 1..1218: mol_type = genomic DNA
atgactgatcgaacgaacgccaatcaaccgctgccactgagccatgatgccagcgttttcgaccgcggcagctgggtagggcgcgtctggttgccggagcaggggccggcggtggtgctggtgaaagccggcgccgtctacgatatcagcacccacgtggcgaccgtctcggcgctgctggaagtggacgatccggtggcctacctgcgtgccttgccgctggccgaacccttgattgcactgccggcattgctgggcaacagcgatcccacacggcgcaccccgcaccagccgtggctgctggcgccgatcgacctgcaagcggtgaaggccgctggtgtgaccttcgccaccagcctgctggagcgtgtggtagaagaacaggccaagggcgacccggccaaggccgacgccatccgtgacaccctggccagccgcatcggcgccgacctgtcgcagatcgtgcccggctcggctcaggccgaagcgctgcgcaaggtgctggtagagcagggcctgtggtcgcagtacctggaggtgggtatcggcccggatgccgaagtgttcaccaaggcccaaccgctgtccgcggttggccacggcgccgacatcggcatccaccccaagtccagctggaacaacccagagccggaagtggtgctggccgtgtcgagcaatggcagcatcaagggcgccatgctcggcaacgacgtcaacctgcgcgacttcgaagggcgtagtgcgttgctgctgtccaaggccaaggacaacaacgcttccactgcactgggcccgctgctgcggttgttcgacgaaagcttcggcctggacgatgtgcgtgctgccgaggtggacctgcgggtggaaggcgaggacggctttatcctctccgggcgcagttccatgcgccagatcagccgtgacccgcaagacctggtgcagcaaaccctcaacgaaaaccaccagtaccctgacggcctggtgctgttcctcggtaccctgttcgcccccaagcaggaccgcgatcagccgggtaacggctttacccacaaaccgggagacgtggtgagcatcagcaacccgcaactgggtaccctgtgcaaccgcgtgaccaccagcgatctggcaccgcagtgggacttcggcctgcgcgcgttgatcgacaacctcggccgacgtggcctgctggaggtcgcggccaccgcccgcccgctttaa

SEQ ID NO: 27 - protein, 310 aa, Cupriavidus necator DSM 13513
MTRTPSPTVYRGVFPVAPTVFDAQGGLDLDGQRRCIDFMIDAGSHGICILANFSEQFVLSDDERNVLMKTVLEHVDGRVPVIVTTTHFSSRLCAERSRAAQDAGAAMVMVMPPYHGATIRVPERSIYEFFATVSDAIDIPIMIQDAPVSGTTLSAPFLARMAREIGNVSYFKIEVPQAAAKLRELIELGGDAIVGPWDGEEAITLMADLEAGATGAMTGAGFPDGIRQILDAWQAGDAELAAQRYQQWLPLINYENRQGWLATSKVLMQAGGVIASDAVRHPLQPMHPATREGLLKIARRLDPLVLRWAR

SEQ ID NO: 28 - DNA, 933 bp, Cupriavidus necator DSM 13513
  source 1..933: mol_type = genomic DNA
atgacccgcaccccatcccccaccgtctaccgcggcgtattcccggtagcgcccaccgtcttcgacgcgcagggcggcctcgacctcgacggccagcgccgctgcatcgacttcatgatcgatgcgggttcgcacggcatctgcatcctggccaacttctccgaacagttcgtgctgagcgacgacgagcgcaacgtgctgatgaagaccgtgctggaacacgtggacggccgcgtgccggtgatcgtcaccaccacgcatttcagctcgcgcctgtgcgccgagcgcagccgcgcggcgcaggatgcgggcgcggccatggtgatggtgatgccgccttaccacggcgccaccatccgcgtgcccgagcgcagcatttacgagttcttcgccacggtctcggatgccatcgacattcccatcatgatccaggacgcgccggtcagcggcaccaccctgagcgcgccgttcctggcgcgcatggcgcgcgagatcggcaatgtgtcgtacttcaagatcgaagtgccgcaggccgcggccaagctgcgcgaactgatcgaactgggcggcgacgccatcgtcggcccctgggacggcgaagaggccatcacgctgatggccgacctggaagcgggcgccaccggcgccatgaccggcgcgggcttccccgacggcatccgccagatcctcgatgcgtggcaggccggcgacgccgaactggccgcgcagcgctaccagcaatggctgccgctgatcaactatgaaaaccggcaaggctggctggccaccagcaaggtgctgatgcaggcaggcggcgtgatcgcatcggacgcggtgcgtcatccgctgcagccgatgcacccggccacccgcgaagggctgctgaagattgcgcgccggctcgatccgctggtgctgcgctgggcccgctga

SEQ ID NO: 29 - protein, 525 aa, Pseudomonas putida DSM 6125
MPLTGNLLIGQRPVTGSRDAIRAIDPTTGQTLEPAYLGGTGEHVAQACALAWAAFDAYRETSLEQRAEFLEAIATQIEALGDALIDRAVIETGLPKARIQGERGRTCTQLRTFARTVRAGEWLDVRIDSALPERQPLPRADLRQRQVALGPVAVFGASNFPLAFSVAGGDTASALAAGCPVVVKAHSAHPGTSELVGQAVAQAVKQCGLPEGVFSLLYGSGREVGIALVSDPRIKAVGFTGSRSGGMALCQAAQARPEPIPVYAEMSSINPVFLFDAALQARAEALAQGFVASLTQGAGQFCTNPGLVIARQGPALQRFITAAAGYVQQGAAQTMLTPGIFSAYQAGIAALADNPHAQAITSGQAGQGPNQCQAQLFVTQAEAFLADPALQAEVFGAASLVVACTDDEQVRQVAEHLEGQLTATLQLDEADIDSARALLPTLERKAGRILVNGWPTGVEVCDAMVHGGPFPATSDARTTSVGTAAILRFLRPVCYQDVPDALLPQALKHGNPLQLRRLLDGKRED

SEQ ID NO: 30 - DNA, 1578 bp, Pseudomonas putida DSM 6125
  source 1..1578: mol_type = genomic DNA
atgcccctcacaggcaacctgctgatcggccagaggccggtaaccggcagccgcgacgccatccgtgccatcgacccaaccaccggtcagacgttggagccggcctacctcggcggcacaggcgaacacgtggcccaggcctgcgcgctggcctgggcggcattcgatgcctaccgcgaaacatcgctcgaacaacgagcagagttccttgaagccatcgccacacagatcgaggccctcggcgatgccctgatcgaccgcgccgtgatcgaaaccggcctgcccaaggcgcgcattcagggcgagcgtggccgtacctgcacccagctacgcacctttgcccgtacagtgcgggccggcgaatggctggacgtgcggatcgacagcgccctgcctgagcgccagcccctcccccgcgctgatttgcgccagcgccaggtggccctggggccagtcgccgtgttcggcgccagcaatttcccgctggccttctcggtggccggtggtgacaccgcgtcggcattggccgctggctgccccgtggtggtcaaggcccacagtgcccaccccggcaccagtgagctggtcggccaggcagtggcgcaagcagtgaagcagtgcggcttaccggagggtgtgttctcgctgctttatggctccggccgcgaagtgggcattgctctggtcagcgacccacgtatcaaggccgttggtttcaccggctcgcgcagcggtggcatggcactgtgccaagccgcccaggcgcgcccggagcccatcccggtgtatgccgaaatgagttcgatcaacccggtgttcctgttcgacgccgccctgcaagcccgtgccgaagcactggcacaaggtttcgtcgcctcgctgacccagggcgccggccagttctgcaccaaccctggcctggtaatcgcccggcaggggccggcactgcagcggttcatcactgcagccgccgggtacgtgcagcagggcgccgcccaaaccatgctcacccctggcattttcagtgcctaccaggccggtatcgcagccctggcagacaacccccatgcccaggccatcaccagtggccaagccggtcagggccccaaccagtgccaggcacagctgttcgtgacccaggccgaagcgtttctcgccgacccggcgttgcaggctgaagtgttcggtgcagcatcgctggtcgttgcctgcaccgacgatgagcaggtccgccaggtagccgaacacctggaaggtcagctgaccgccaccctgcaactggacgaggccgacatcgacagcgctcgcgccctgctccccacccttgagcgcaaggccgggcgtattctggtcaatggctggccgaccggcgtcgaggtgtgcgatgccatggtccacggcgggccgttcccggccacttccgatgcccgtaccacctcggtgggcacggcggcgatcctgcgtttcctgcgcccggtttgctatcaggacgtccccgatgcgctgctgccgcaggcattgaaacacggcaacccgctgcagctgcggcgcctgcttgatggtaaacgggaagactga

SEQ ID NO: 31 - protein, 266 aa, Picrophilus torridus
MITPLDAHGNIDYNATNILIKYLEGINVDYLFPMGSTGVFPYFTLKERKDFLKFVRENSKKPIMAGVGSSSINEVNELMKFSMDIGIEAAVLMPPYYIKLNQEAIYHYYKEILSSNDMDLLIYNIPQFTNKIDPETVKNLKSEFSSVKGVKDSSADIRGFMEMLSLSDDDFAVFQGQDDLLFTSLELGASGGVCGTTNFSDGIVRLYHEYKNNREMALKIEKNDVIPLMKKLGKYQFPNAYYEYFYKKNNINGGYRPPMYRVGIEI

SEQ ID NO: 32 - DNA, 801 bp, Picrophilus torridus
  source 1..801: mol_type = other DNA
atgattaccccgctggacgcacacggcaacatcgactataacgcaacgaacattctgatcaaatacctggaaggcatcaacgtggactacctgttcccgatgggctctaccggtgtgtttccgtatttcacgctgaaagaacgtaaagactttctgaaattcgttcgcgaaaacagtaaaaaaccgatcatggctggcgtcggtagctctagtatcaacgaagtgaacgaactgatgaaattcagcatggatatcggtatcgaagcggccgtgctgatgccgccatattacattaaactgaaccaggaagcaatctaccattactacaaagaaatcctgtcctcaaatgacatggatctgctgatttacaacatcccgcaatttaccaataaaatcgatccggaaacggtcaaaaacctgaaatctgaatttagcagcgtgaaaggtgttaaagactctagtgcagatattcgtggctttatggaaatgctgtccctgtcagatgacgattttgctgttttccagggtcaagacgatctgctgtttacctcgctggaactgggtgccagcggcggtgtttgtggtaccacgaattttagcgacggcatcgtccgtctgtatcacgaatacaaaaacaatcgcgaaatggccctgaaaattgagaaaaacgatgttatcccgctgatgaaaaaactgggcaaatatcagtttccgaatgcatattacgaatatttctacaagaaaaacaatatcaatggcggctaccgtccgccgatgtatcgcgttggcatcgaaatctaa

SEQ ID NO: 33 - protein, 258 aa, Sphingomonas sp.
MFSDLKGKRILITGSTEGIGMATAIELARYGAVVGLNSHVDPADPALLLGKLREAGGDGAFFRADITKTAECQRLVSAFVERFDGIDVLINNAGGLAGRSNLENIDDAFYDRVMDLNGRSVLMMTKFAIPHLRASAKASGTTSAVISTGSIAAREGGGIGAGVYAASKAWLHDIHRNWVKEFTKDSIRFNIVAPGTVDTAFHADKSDELKTRIANSIPMGRFGTVQELAPAYVFFASHAASGYITGQILDVNGGQICP

SEQ ID NO: 34 - DNA, 777 bp, Sphingomonas sp.
  source 1..777: mol_type = other DNA
atgttcagcgacctgaaaggtaaacgtattctgattaccggtagcaccgaaggtattggtatggcaaccgcaattgaactggcacgttatggtgcagttgttggtctgaatagccatgttgatccggcagatcctgcactgctgctgggtaaactgcgtgaagccggtggtgatggtgcattttttcgtgcagatatcaccaaaaccgcagaatgtcagcgtctggttagcgcatttgttgaacgttttgatggtattgatgtgctgattaacaatgccggtggtctggcaggtcgtagcaatctggaaaatattgatgatgccttttatgaccgtgtgatggatctgaatggtcgtagcgttctgatgatgaccaaatttgcaattccgcatctgcgtgcaagcgcaaaagcaagcggtacaaccagcgcagttattagcaccggtagtattgcagcacgtgaaggtggtggtattggtgccggtgtttatgcagcaagcaaagcatggctgcatgatattcatcgtaattgggtgaaagagttcaccaaagatagcatccgttttaacattgttgcaccgggtacagttgataccgcatttcatgcagataaaagcgacgaactgaaaacccgtattgcaaatagcattccgatgggtcgttttggcaccgttcaagagctggcaccagcctatgttttttttgcaagccatgccgcaagcggttatatcaccggtcagattctggatgttaatggtggtcagatttgtccgtaa

SEQ ID NO: 35 - protein, 1231 aa, Mycobacterium tuberculosis H37Rv
MANISSPFGQNEWLVEEMYRKFRDDPSSVDPSWHEFLVDYSPEPTSQPAAEPTRVTSPLVAERAAAAAPQAPPKPADTAAAGNGVVAALAAKTAVPPPAEGDEVAVLRGAAAAVVKNMSASLEVPTATSVRAVPAKLLIDNRIVINNQLKRTRGGKISFTHLLGYALVQAVKKFPNMNRHYTEVDGKPTAVTPAHTNLGLAIDLQGKDGKRSLVVAGIKRCETMRFAQFVTAYEDIVRRARDGKLTTEDFAGVTISLTNPGTIGTVHSVPRLMPGQGAIIGVGAMEYPAEFQGASEERIAELGIGKLITLTSTYDHRIIQGAESGDFLRTIHELLLSDGFWDEVFRELSIPYLPVRWSTDNPDSIVDKNARVMNLIAAYRNRGHLMADTDPLRLDKARFRSHPDLEVLTHGLTLWDLDRVFKVDGFAGAQYKKLRDVLGLLRDAYCRHIGVEYAHILDPEQKEWLEQRVETKHVKPTVAQQKYILSKLNAAEAFETFLQTKYVGQKRFSLEGAESVIPMMDAAIDQCAEHGLDEVVIGMPHRGRLNVLANIVGKPYSQIFTEFEGNLNPSQAHGSGDVKYHLGATGLYLQMFGDNDIQVSLTANPSHLEAVDPVLEGLVRAKQDLLDHGSIDSDGQRAFSVVPLMLHGDAAFAGQGVVAETLNLANLPGYRVGGTIHIIVNNQIGFTTAPEYSRSSEYCTDVAKMIGAPIFHVNGDDPEACVWVARLAVDFRQRFKKDVVIDMLCYRRRGHNEGDDPSMTNPYVYDVVDTKRGARKSYTEALIGRGDISMKEAEDALRDYQGQLERVFNEVRELEKHGVQPSESVESDQMIPAGLATAVDKSLLARIGDAFLALPNGFTAHPRVQPVLEKRREMAYEGKIDWAFGELLALGSLVAEGKLVRLSGQDSRRGTFSQRHSVLIDRHTGEEFTPLQLLATNSDGSPTGGKFLVYDSPLSEYAAVGFEYGYTVGNPDAVVLWEAQFGDFVNGAQSIIDEFISSGEAKWGQLSNVVLLLPHGHEGQGPDHTSARIERFLQLWAEGSMTIAMPSTPSNYFHLLRRHALDGIQRPLIVFTPKSMLRHKAAVSEIKDFTEIKFRSVLEEPTYEDGIGDRNKVSRILLTSGKLYYELAARKAKDNRNDLAIVRLEQLAPLPRRRLRETLDRYENVKEFFWVQEEPANQGAWPRFGLELPELLPDKLAGIKRISRRAMSAPSSGSSKVHAVEQQEILDEAFG

SEQ ID NO: 36 - DNA, 3696 bp, Mycobacterium tuberculosis H37Rv
  source 1..3696: mol_type = genomic DNA
atggccaacataagttcaccattcgggcaaaacgaatggctggtcgaagagatgtaccgcaagttccgcgacgacccctcctcggtcgatcccagctggcacgagttcctggttgactacagccccgaacccacctcccaaccagctgccgaaccaacccgggttacctcgccactcgttgccgagcgggccgctgcggccgccccgcaggcaccccccaagccggccgacaccgcggccgcgggcaacggcgtggtcgccgcactggccgccaaaactgccgttcccccgccagccgaaggtgacgaggtagcggtgctgcgcggcgccgccgcggccgtcgtcaagaacatgtccgcgtcgttggaggtgccgacggcgaccagcgtccgggcggtcccggccaagctactgatcgacaaccggatcgtcatcaacaaccagttgaagcggacccgcggcggcaagatctcgttcacgcatttgctgggctacgccctggtgcaggcggtgaagaaattcccgaacatgaaccggcactacaccgaagtcgacggcaagcccaccgcggtcacgccggcgcacaccaatctcggcctggcgatcgacctgcaaggcaaggacgggaagcgttccctggtggtggccggcatcaagcggtgcgagaccatgcgattcgcgcagttcgtcacggcctacgaagacatcgtacgccgggcccgcgacggcaagctgaccactgaagactttgccggcgtgacgatttcgctgaccaatcccggaaccatcggcaccgtgcattcggtgccgcggctgatgcccggccagggcgccatcatcggcgtgggcgccatggaataccccgccgagtttcaaggcgccagcgaggaacgcatcgccgagctgggcatcggcaaattgatcactttgacctccacctacgaccaccgcatcatccagggcgcggaatcgggcgacttcctgcgcaccatccacgagttgctgctctcggatggcttctgggacgaggtcttccgcgaactgagcatcccatatctgccggtgcgctggagcaccgacaaccccgactcgatcgtcgacaagaacgctcgcgtcatgaacttgatcgcggcctaccgcaaccgcggccatctgatggccgataccgacccgctgcggttggacaaagctcggttccgcagtcaccccgacctcgaagtgctgacccacggcctgacgctgtgggatctcgatcgggtgttcaaggtcgacggctttgccggtgcgcagtacaagaaactgcgcgacgtgctgggcttgctgcgcgatgcctactgccgccacatcggcgtggagtacgcccatatcctcgaccccgaacaaaaggagtggctcgaacaacgggtcgagaccaagcacgtcaaacccactgtggcccaacagaaatacatcctcagcaagctcaacgccgccgaggcctttgaaacgttcctacagaccaagtacgtcggccagaagcggttctcgctggaaggcgccgaaagcgtgatcccgatgatggacgcggcgatcgaccagtgcgctgagcacggcctcgacgaggtggtcatcgggatgccgcaccggggccggctcaacgtgctggccaacatcgtcggcaagccgtactcgcagatcttcaccgagttcgagggcaacctgaatccgtcgcaggcgcacggctccggtgacgtcaagtaccacctgggcgccaccgggctgtacctgcagatgttcggcgacaacgacattcaggtgtcgctgaccgccaacccgtcgcatctggaggccgtcgacccggtgctggagggattggtgcgggccaagcaggatctgctcgaccacggaagcatcgacagcgacggccaacgggcgttctcggtggtgccgctgatgttgcatggcgatgccgcgttcgccggtcagggtgtggtcgccgagacgctgaacctggcgaatctgccgggctaccgcgtcggcggcaccatccacatcatcgtcaacaaccagatcggcttcaccaccgcgcccgagtattccaggtccagcgagtactgcaccgacgtcgcaaagatgatcggggcaccgatctttcacgtcaacggcgacgacccggaggcgtgtgtctgggtggcgcggttggcggtggacttccgacaacggttcaagaaggacgtcgtcatcgacatgctgtgctaccgccgccgcgggcacaacgagggtgacgacccgtcgatgaccaacccctacgtgtacgacgtcgtcgacaccaagcgcggggcccgcaaaagctacaccgaagccctgatcggacgtggcgacatctcgatgaaggaggccgaggacgcgctgcgcgactaccagggccagctggaacgggtgttcaacgaagtgcgcgagctggagaagcacggtgtgcagccgagcgagtcggtcgagtccgaccagatgattcccgcggggctggccactgcggtggacaagtcgctgctggcccggatcggcgatgcgttcctcgccttgccgaacggcttcaccgcgcacccgcgagtccaaccggtgctggagaagcgccgggagatggcctatgaaggcaagatcgactgggcctttggcgagctgctggcgctgggctcgctggtggccgaaggcaagctggtgcgcttgtcggggcaggacagccgccgcggcaccttctcccagcggcattcggttctcatcgaccgccacactggcgaggagttcacaccactgcagctgctggcgaccaactccgacggcagcccgaccggcggaaagttcctggtctacgactcgccactgtcggagtacgccgccgtcggcttcgagtacggctacactgtgggcaatccggacgccgtggtgctctgggaggcgcagttcggcgacttcgtcaacggcgcgcagtcgatcatcgacgagttcatcagctccggtgaggccaagtggggccaattgtccaacgtcgtgctgctgttaccgcacgggcacgaggggcagggacccgaccacacttctgcccggatcgaacgcttcttgcagttgtgggcggaaggttcgatgaccatcgcgatgccgtcgactccgtcgaactacttccacctgctacgccggcatgccctggacggcatccaacgcccgctgatcgtgttcacgcccaagtcgatgttgcgtcacaaggccgccgtcagcgaaatcaaggacttcaccgagatcaagttccgctcagtgctggaggaacccacctatgaggacggcatcggagaccgcaacaaggtcagccggatcctgctgaccagtggcaagctgtattacgagctggccgcccgcaaggccaaggacaaccgcaatgacctcgcgatcgtgcggcttgaacagctcgccccgctgcccaggcgtcgactgcgtgaaacgctggaccgctacgagaacgtcaaggagttcttctgggtccaagaggaaccggccaaccagggtgcgtggccgcgattcgggctcgaactacccgagctgctgcctgacaagttggccgggatcaagcgaatctcgcgccgggcgatgtcagccccgtcgtcaggctcgtcgaaggtgcacgccgtcgaacagcaggagatcctcgacgaggcgttcggctga

SEQ ID NO: 37 - protein, 254 aa, Rhodobacter sphaeroides D
MDYRTVFRLDGACAAVTGAGSGIGLEICRAFAASGARLILIDREAAALDRAAQELGAAVAARIVADVTDAEAMTAAAAEAEAVAPVSILVNSAGIARLHDALETDDATWRQVMAVNVDGMFWASRAFGRAMVARGAGAIVNLGSMSGTIVNRPQFASSYMASKGAVHQLTRALAAEWAGRGVRVNALAPGYVATEMTLKMRERPELFETWLDMTPMGRCGEPSEIAAAALFLASPAASYVTGAILAVDGGYTVW

SEQ ID NO: 38 - DNA, 765 bp, Rhodobacter sphaeroides D
  source 1..765: mol_type = other DNA
atggattatcgtacggtgtttcgcttagatggtgcttgtgccgcagtgacgggtgccgggtcgggaattggactggagatttgtcgcgcatttgctgcaagcggtgcacgcctgattctgattgaccgcgaagcagcagcgctggatcgtgccgctcaagaactgggtgccgcagtcgccgcccgtattgtagcggatgtaacagacgctgaagcaatgacggcggccgcagcagaagctgaggcggtagcacccgtttcaattcttgttaacagcgccggtattgcacgtttacatgacgccctggaaacggatgatgctacgtggcgtcaagttatggccgtgaacgtcgatggtatgttttgggcatcacgtgcgtttggtcgtgcgatggttgcccgtggcgcgggcgcgattgtcaatcttggttctatgagcggtacaattgttaatcgtccccaatttgcgtcatcatatatggcaagcaaaggtgcagtacaccaattaacccgtgccctggcagcagagtgggccggtcgtggggttcgcgttaacgccttagctccagggtacgtagccacggaaatgacccttaaaatgcgtgaacgtccagaattgtttgaaacatggctggatatgacccctatgggacgttgtggtgaaccgagtgaaattgcagccgctgccttatttctggctagtcccgcagcttcatacgtgactggtgcaattctggctgttgatggtgggtatactgtttggtaa

SEQ ID NO: 39 - protein, 558 aa, Acetobacter pasteurianus
MTYTVGMYLAERLVQIGLKHHFAVAGDYNLVLLDQLLLNKDMKQIYCCNELNCGFSAEGYARSNGAAAAVVTFSVGAISAMNALGGAYAENLPVILISGAPNSNDQGTGHILHHTIGKTDYSYQLEMARQVTCAAESITDAHSAPAKIDHVIRTALRERKPAYLDIACNIASEPCVRPGPVSSLLSEPEIDHTSLKAAVDATVALLEKSASPVMLLGSKLRAANALAATETLADKLQCAVTIMAAAKGFFPEDHAGFRGLYWGEVSNPGVQELVETSDALLCIAPVFNDYSTVGWSAWPKGPNVILAEPDRVTVDGRAYDGFTLRAFLQALAEKAPARPASAQKSSVPTCSLTATSDEAGLTNDEIVRHINALLTSNTTLVAETGDSWFNAMRMTLPRGARVELEMQWGHIGWSVPSAFGNAMGSQDRQHVVMVGDGSFQLTAQEVAQMVRYELPVIIFLINNRGYVIEIAIHDGPYNYIKNWDYAGLMEVFNAGEGHGLGLKATTPKELTEAIARAKANTRGPTLIECQIDRTDCTDMLVQWGRKVASTNARKTTLA

SEQ ID NO: 40 - DNA, 1674 bp, Acetobacter pasteurianus
  source 1..1674: mol_type = other DNA
atgacatacactgtaggaatgtatctagctgagcgcctggttcaaatcggcctgaagcaccactttgcagtgggcggtgactataatctggtgctgttggaccagttgctgttgaacaaagatatgaaacaaatttactgctgcaatgagctgaactgcggtttctccgcggagggctacgcccgtagcaacggcgcagcggcggccgtggtgaccttttcagtgggtgccatcagcgcaatgaacgctctgggtggtgcgtacgccgagaatttaccggtgatcctgatcagtggtgctccgaacagcaatgatcaaggtacaggccacattctgcatcacaccattggcaaaaccgactacagctatcagttggagatggcgcgtcaggttacgtgcgcagcggagtccattaccgacgcgcatagcgctccggcaaagatcgaccacgtcattcgtaccgccctgcgtgaacgtaagccggcttacctggacatcgcgtgtaatattgcatcggagccgtgtgttcgtccgggcccggttagcagcctgctgagcgagccggaaatcgaccacacctctttgaaggcagcggtggatgcgaccgtcgcgctgctgaagaatcgtccggctccggtcatgctgcttggcagcaaactgagagccgcgaacgcgctggcggcgactgaaacgctggctgataaattacaatgtgcagttaccattatggcagcggcgaagggcttcttcccggaagatcatgcaggtttccgcggtctgtattggggtgaggtttctaacccgggtgttcaagagttggttgaaacctccgacgcgctgctttgcattgcgccagtgttcaacgactacagcaccgttggctggtccggcatgccgaaaggtccgaatgttatcctggcggagccagatcgtgtcactgtcgatggtcgcgcgtacgacggcttcaccctgcgtgcgttcttgcaagcactggcggagaaagcgccggctcgtcctgcgagcgcacagaaaagcagcgtaccaacgtgcagcctgaccgcgacgtctgacgaagcaggcttgacgaatgatgaaattgttcgtcatatcaacgcgctgctcacttcgaataccaccttggtcgctgaaaccggtgatagctggtttaacgccatgcgtatgaccctagccggcgcacgtgtagagctggagatgcagtggggtcacatcggttggtccgttccgagcgcgtttggtaacgcgatgggttctcaggatcgccagcatgtcgtgatggtgggcgacggcagttttcagttgactgcgcaagaagtggcccaaatggtgcgttatgaacttccggttattatctttctgatcaacaaccgcggatacgtgatcgagatcgctatccacgatggtccgtataactatattaaaaactgggattacgctggtctgatggaagtgttcaacgcaggcgaaggtcatgggctgggcctgaaggctaccaccccgaaagaactcacggaagcaatcgcgagggcgaaggccaatactcgtggtccgaccctcattgagtgccagatcgaccgcaccgactgtaccgacatgctggttcagtggggtcgtaaggtggcgtcaacgaacgctcgcaagaccactctcgcctaa